European Patent Application EP 4 552 639 A1, published May 14, 2025. Title: Compounds for use in the treatment of gastrointestinal stromal tumor (GIST). Applicant: Universität Duisburg-Essen. The sequence listing filed with the application follows.

SEQUENCE LISTING (30 sequences)

SEQ ID NO: 1 - RNA, 20 nt, synthetic construct
  source 1..20: mol_type = other RNA
atgaatattgtgaatctact

SEQ ID NO: 2 - RNA, 20 nt, synthetic construct
  source 1..20: mol_type = other RNA
tgtgattaccaaggtaactc

SEQ ID NO: 3 - RNA, 20 nt, synthetic construct
  source 1..20: mol_type = other RNA
agaatcattcttgatgtctc

SEQ ID NO: 4 - RNA, 20 nt, synthetic construct
  source 1..20: mol_type = other RNA
gattctaattatgtggttaa

SEQ ID NO: 5 - RNA, 21 nt, synthetic construct
  source 1..21: mol_type = other RNA
aagctaatacgactcactata

SEQ ID NO: 6 - RNA, 43 nt, synthetic construct
  source 1..43: mol_type = other RNA
nnnnnnnnnnnnnnnnnnnngtttaagagctatgctggaaaca

SEQ ID NO: 7 - RNA, 92 nt, synthetic construct
  source 1..92: mol_type = other RNA
aaaaaagcaccgactcggtgccactttttcaagttgataacggactagccttatttaaacttgctatgctgtttccagcatagctcttaaac

SEQ ID NO: 8 - DNA, 105 bp, synthetic construct
  source 1..105: mol_type = other DNA
  misc_difference 104^105: note = the indicated nucleotides are linked via a PTO (phosphorothioate) base link
acagacaataaaaggcagcttggacacggctttacctccaatggtgcaggctccgagaagattcgcaatattcatgtgattaccaaggtaactcaggactttgag

SEQ ID NO: 9 - DNA, 105 bp, synthetic construct
  source 1..105: mol_type = other DNA
  misc_difference 104^105: note = the indicated nucleotides are linked via a PTO (phosphorothioate) base link
gccagaaatatcctccttactcatggtcggatcacaaagatttgtgattttggtctagcaagggccatcaagaatgattctaattatgtggttaaaggaaacgtg

SEQ ID NO: 10 - RNA, 20 nt, synthetic construct
  source 1..20: mol_type = other RNA
cgaatcatgcatgatgtctc

SEQ ID NO: 11 - RNA, 20 nt, synthetic construct
  source 1..20: mol_type = other RNA
tgaagataatgactcacctg

SEQ ID NO: 12 - RNA, 20 nt, synthetic construct
  source 1..20: mol_type = other RNA
atcacagagtattgcttcta

SEQ ID NO: 13 - RNA, 20 nt, synthetic construct
  source 1..20: mol_type = other RNA
accgcgatgagaggcgctcg

SEQ ID NO: 14 - DNA, 95 bp, synthetic construct
  source 1..95: mol_type = other DNA
  misc_difference 94^95: note = the indicated nucleotides are linked via a PTO (phosphorothioate) base link
tcctcctggcacaaggaaaaattgtgaagatctgtgactttggcctggcaagagtcatcatgcatgattcgaactatgtgtcgaaaggcagtgta

SEQ ID NO: 15 - DNA, 100 bp, synthetic construct
  source 1..100: mol_type = other DNA
  misc_difference 99^100: note = the indicated nucleotides are linked via a PTO (phosphorothioate) base link
caagctctcatgtctgaactgaagataatgactcacctggagccacatttaaacattgcaaacttgctgggagcctgcaccaagtcaggtgggctcactg

SEQ ID NO: 16 - DNA, 105 bp, synthetic construct
  source 1..105: mol_type = other DNA
  misc_difference 104^105: note = the indicated nucleotides are linked via a PTO (phosphorothioate) base link
cttcattttcatacccatctcctaacggcttttgtccccatagggccgatttacatcatcatagagtattgcttctatggagatttggtcaactatttgcataag

SEQ ID NO: 17 - DNA, 99 bp, synthetic construct
  source 1..99: mol_type = other DNA
  misc_difference 98^99: note = the indicated nucleotides are linked via a PTO (phosphorothioate) base link
gtccccataggccccatttacatcatcacagagtattgcttctatagagatttagtcaactatttgcataagaatagggatagcttcctgagccaccac

SEQ ID NO: 18 - DNA, 25 bp, synthetic construct
  source 1..25: mol_type = other DNA
cagtggaaggttgatcacaaatggg

SEQ ID NO: 19 - RNA, 20 nt, synthetic construct
  source 1..20: mol_type = other RNA
tgtaaggcttacaacgatgt

SEQ ID NO: 20 - DNA, 119 bp, synthetic construct
  source 1..119: mol_type = other DNA
  misc_difference 1^2: note = the indicated nucleotides are linked via a PTO (phosphorothioate) base link
  misc_difference 2^3: note = the indicated nucleotides are linked via a PTO (phosphorothioate) base link
  misc_difference 118^119: note = the indicated nucleotides are linked via a PTO (phosphorothioate) base link
  misc_difference 117^118: note = the indicated nucleotides are linked via a PTO (phosphorothioate) base link
agtgcattcaagcacaatggcacggttgaatgtaaggcttacaatgacgtgggcaagacttctgcctatgcctattttaactttgcatttaaaggtaacaacaaaggtatatttctttt

SEQ ID NO: 21 - RNA, 20 nt, synthetic construct
  source 1..20: mol_type = other RNA
gtggaaggttgatcacaaat

SEQ ID NO: 22 - DNA, 155 bp, synthetic construct
  source 1..155: mol_type = other DNA
  misc_difference 1^2: note = the indicated nucleotides are linked via a PTO (phosphorothioate) base link
  misc_difference 2^3: note = the indicated nucleotides are linked via a PTO (phosphorothioate) base link
  misc_difference 154^155: note = the indicated nucleotides are linked via a PTO (phosphorothioate) base link
  misc_difference 153^154: note = the indicated nucleotides are linked via a PTO (phosphorothioate) base link
tttccctttctccccacagaaacccatgtatgaagtacagtggaaggttgttgaggagataaacgggaataattatgtttacatagacccaacacaacttccttatgatcacaaatgggagtttcccagaaacaggctgagttttggtcagtatg

SEQ ID NO: 23 - RNA, 20 nt, synthetic construct
  source 1..20: mol_type = other RNA
atgaatattgtgaatctact

SEQ ID NO: 24 - DNA, 88 bp, synthetic construct
  source 1..88: mol_type = other DNA
  misc_difference 1^2: note = the indicated nucleotides are linked via a PTO (phosphorothioate) base link
  misc_difference 87^88: note = the indicated nucleotides are linked via a PTO (phosphorothioate) base link
  misc_difference 86^87: note = the indicated nucleotides are linked via a PTO (phosphorothioate) base link
ctcaaagtcctgagttaccttggtaatcacatgaatattgcgaaccttcttggagcctgcaccattggaggtaaagccgtgtccaagc

SEQ ID NO: 25 - RNA, 20 nt, synthetic construct
  source 1..20: mol_type = other RNA
agaatcattcttgatgtctc

SEQ ID NO: 26 - DNA, 102 bp, synthetic construct
  source 1..102: mol_type = other DNA
  misc_difference 1^2: note = the indicated nucleotides are linked via a PTO (phosphorothioate) base link
  misc_difference 101^102: note = the indicated nucleotides are linked via a PTO (phosphorothioate) base link
  misc_difference 100^101: note = the indicated nucleotides are linked via a PTO (phosphorothioate) base link
cagaaatatcctccttactcatggtcggatcacaaagattggtgattttggtctagctagagacatcaagaatgattctaattatgtggttaaaggaaacgt

SEQ ID NO: 27 - RNA, 20 nt, synthetic construct
  source 1..20: mol_type = other RNA
caagaatgattctaattatg

SEQ ID NO: 28 - DNA, 94 bp, synthetic construct
  source 1..94: mol_type = other DNA
  misc_difference 1^2: note = the indicated nucleotides are linked via a PTO (phosphorothioate) base link
  misc_difference 93^94: note = the indicated nucleotides are linked via a PTO (phosphorothioate) base link
  misc_difference 92^93: note = the indicated nucleotides are linked via a PTO (phosphorothioate) base link
aagatttgtgattttggtctagccagagacatcaagaatgcttctaattatgtcgttaaaggaaacgtgagtacccattctctgcttgacagtc

SEQ ID NO: 29 - DNA, 101 bp, synthetic construct
  source 1..101: mol_type = other DNA
  misc_difference 100^101: note = the indicated nucleotides are linked via a PTO (phosphorothioate) base link
cacaaagatttgtgattttggtctagccagagacatcaagaattattctaattatgtcgttaaaggaaacgtgagtacccattctctgcttgacagtcctg

SEQ ID NO: 30 - DNA, 110 bp, synthetic construct
  source 1..110: mol_type = other DNA
  misc_difference 109^110: note = the indicated nucleotides are linked via a PTO (phosphorothioate) base link
tactcatggtcggatcacaaagatttgtgattttggtctagccagagacatcaagaatgattctaagtatgtggttaaaggaaacgtgagtacccattctctgcttgaca